European Patent Application EP 4 692 343 A1, published February 11, 2026. Title: A chinese hamster artificial chromosome vector or a fragment thereof, and a cell derived from mammal comprising the same. Applicant: 株式会社Trans Chromosomics. Application JP. The sequence listing filed with the application follows.

SEQUENCE LISTING (16 sequences)

SEQ ID NO: 1 - DNA, 25 bp, synthetic construct
  misc_feature 1..25: note = primer
  source 1..25: mol_type = other DNA
ataagcgggtaaaatcccgactatg

SEQ ID NO: 2 - DNA, 25 bp, synthetic construct
  misc_feature 1..25: note = primer
  source 1..25: mol_type = other DNA
gcatttggcgtatccactgactatc

SEQ ID NO: 3 - DNA, 28 bp, synthetic construct
  misc_feature 1..28: note = primer
  source 1..28: mol_type = other DNA
aatggaagtagcacgtctcactagtctc

SEQ ID NO: 4 - DNA, 30 bp, synthetic construct
  misc_feature 1..30: note = primer
  source 1..30: mol_type = other DNA
gcgacgatacaagtcaggttgccagctgcc

SEQ ID NO: 5 - DNA, 30 bp, synthetic construct
  misc_feature 1..30: note = primer
  source 1..30: mol_type = other DNA
ggtagccaacgctatgtcctgatagcggtc

SEQ ID NO: 6 - DNA, 20 bp, synthetic construct
  misc_feature 1..20: note = primer
  source 1..20: mol_type = other DNA
taagggattttgccgatttc

SEQ ID NO: 7 - DNA, 24 bp, synthetic construct
  misc_feature 1..24: note = primer
  source 1..24: mol_type = other DNA
agacaaaccacgaagacacaggtc

SEQ ID NO: 8 - DNA, 22 bp, synthetic construct
  misc_feature 1..22: note = primer
  source 1..22: mol_type = other DNA
tcctttgcaacccaggccgttc

SEQ ID NO: 9 - DNA, 23 bp, synthetic construct
  misc_feature 1..23: note = primer
  source 1..23: mol_type = other DNA
agctgaccctgaagttcatctgc

SEQ ID NO: 10 - DNA, 24 bp, synthetic construct
  misc_feature 1..24: note = primer
  source 1..24: mol_type = other DNA
aacttgatgttgacgttgtaggcg

SEQ ID NO: 11 - DNA, 25 bp, synthetic construct
  misc_feature 1..25: note = primer
  source 1..25: mol_type = other DNA
catggccatcatcaaggagttcatg

SEQ ID NO: 12 - DNA, 26 bp, synthetic construct
  misc_feature 1..26: note = primer
  source 1..26: mol_type = other DNA
ccggatcggacgattgcgtcgcatcg

SEQ ID NO: 13 - DNA, 1566 bp, Homo sapiens
  source 1..1566: mol_type = unassigned DNA
atgaaacatctgtggttcttccttctcctggtggcagctcccagatgggtcctgtcccaggtgcagctgcaggagtcgggcccaggactggtgaagccttcggagaccctgtccctcacctgcactgtctctggtggctccatcagtagttactactggagctggatccggcagcccccagggaagggactggagtggattgggtatatctattacagtgggtacaccaagtacaacccctccctcaagagtcgagtcaccatatcaatagacacgtccaagaaccagttctccctgaagctgagctctgtgaccgctgcggacacggccgtgtattactgtgcgagagaagggggtatgattcggggagttattggctactactacggtatggacgtctggggccaagggaccacggtcaccgtctcctcagcttccaccaagggcccatcggtcttccccctggcgccctgctccaggagcacctctgggggcacagcggccctgggctgcctggtcaaggactacttccccgaaccggtgacggtgtcgtggaactcaggcgccctgaccagcggcgtgcacaccttcccggctgtcctacagtcctcaggactctactccctcagcagcgtggtgaccgtgccctccagcagcttgggcacccagacctacacctgcaacgtgaatcacaagcccagcaacaccaaggtggacaagagagttgagctcaaaaccccacttggtgacacaactcacacatgcccacggtgcccagagcccaaatcttgtgacacacctcccccgtgcccacggtgcccagagcccaaatcttgtgacacacctcccccatgcccacggtgcccagagcccaaatcttgtgacacacctcccccgtgcccaaggtgcccagcacctgaactcctgggaggaccgtcagtcttcctcttccccccaaaacccaaggatacccttatgatttcccggacccctgaggtcacgtgcgtggtggtggacgtgagccacgaagaccccgaggtccagttcaagtggtacgtggacggcgtggaggtgcataatgccaagacaaagctgcgggaggagcagtacaacagcacgttccgtgtggtcagcgtcctcaccgtcctgcaccaggactggctgaacggcaaggagtacaagtgcaaggtctccaacaaagccctcccagcccccatcgagaaaaccatctccaaaaccaaaggacagccccgagaaccacaggtgtacaccctgcccccatcccgggaggagatgaccaagaaccaggtcagcctgacctgcctggtcaaaggcttctaccccagcgacatcgccgtggagtgggagagcaatgggcagccggagaacaactacaacaccacgcctcccatgctggactccgacggctccttcttcctctacagcaagctcaccgtggacaagagcaggtggcagcaggggaacatcttctcatgctccgtgatgcatgaggctctgcacaaccgctacacgcagaagagcctctccctgtctccgggtaaatga

SEQ ID NO: 14 - DNA, 759 bp, Homo sapiens
  source 1..759: mol_type = unassigned DNA
atgggggagctacaacaggcaggcaggggcagcaagatggtgttgcagacccaggtcttcatttctctgttgctctggatctctggtgcctacggggacatcgtgatgacccagtctccagactccctggctgtgtctctgggcgagagggccaccatcaactgcaagtccagccagagtgttttatacagctccaacaataagaactacttagtttggtaccagcagaaaccaggacagcctcctaagctgctcatttactgggcatctacccgggaatccggggtccctgaccgattcagtggcagcgggtctgggacagatttcactctcaccatcagcagcctgcaggctgaagatgtggcagtttattactgtcagcaatattatagtactccgtacacttttggccaggggaccaagctggagatcaaacgaactgtggctgcaccatctgtcttcatcttcccgccatctgatgagcagttgaaatctggaactgcctctgttgtgtgcctgctgaataatttctatcccagagaggccaaagtacagtggaaggtggataacgccctccaatcgggtaactcccaggagagtgtcacagagcaggacagcaaggacagcacctacagcctcagcagcaccctgacgctgagcaaagcagactacgagaaacacaaactctacgcctgcgaagtcacccatcagggcctgagctcgcccgtcacaaagagcttcaacaggggagagtgttag

SEQ ID NO: 15 - DNA, 1047 bp, Cricetulus griseus
  source 1..1047: mol_type = unassigned DNA
atgaccgagatgagcttcctgaacagcgaagtgttggctggggacttgatgtcccccttcgaccagtcgggtttgggggctgaagaaagcctagggctcttagatgactacctggaggtggccaagcacttcaaacctcatgggttctccagcgacaaggctaaggcgggctcctccgaatggctggctgtggatgggttggtcagtgcctcagacaccggcaaggaggatgcattctccgggacagactggatgttggagaaaatggatcttaaagagtttgactttgatgctctgtttcgaatggatgacctggataccatgccagatgagcttttggccacgttggatgacacatgtgatctttttgcccctctagtccaagagactaacaaggagcccatgacagtgaacccaattggccatctcccagaaagtgcaacaaaaatagaccaggttgccccctttgcattcttgcaaccttttccctgttccccaggggtcctgtcttccactccagatcattccttcagtttagagttaggcagtgaagttgatatctctgaaggagacaggaagcctgactctgcttatattactctaatcccccagtgtgtaaaggatgaagacaccccctcagataatgacagtggcatctgtatgagccctgagtcctacctgggctccccccagcatagcccctccacctccaggggatcaccaagcagtctgccctctccagttgttacccgtgggtcaccaagacccaaaccttatgacccccctggagttactttaacagctaaagtgaaaattgaaaagttggataagaagctaaaaaaaatggagcaaaacaagacagcagccactagataccgacagaagaagcgggctgaacaggaagccctgacaggcgagtgtagagagctagaaaagaagaatgaagctctaaaagagaaggcagattctcttgccaaagagatccaatatctgaaagatctgatagaagaggtccggaaggcaagggggaagaagagagctccctag

SEQ ID NO: 16 - DNA, 1047 bp, Cricetulus griseus
  source 1..1047: mol_type = unassigned DNA
atgaccgagatgagcttcctgaacagcgaagtgttggctggggacttgatgtcccccttcgaccagtcgggtttgggggctgaagaaagcctggggctcttagatgactacctggaggtggccaagcacttcaaacctcatgggttctccagcgacaaggctaaggcgggctcctccgaatggctggctgtggatgggttggtcagtgcctcagacaccggcaaggaggatgcattctccgggacagactggatgttggagaaaatggatcttaaagagtttgactttgatgctctgtttcgaatggatgacctggataccatgccagatgagcttttggccacgttggatgacacatgtgatctttttgcccctctagtccaagagactaacaaggagcccatgacagtgaacccaattggccatctcccagaaagtgcaacaaaaatagaccaggttgccccctttgcattcttgcaaccttttccctgttccccaggggtcctgtcttccactccagatcattccttcagtttagagttaggcagtgaagttgatatctctgaaggagacaggaagcctgactctgcttatattactctaatcccccagtgtgtaaaggatgaagacaccccctcagataatgacagtggcatctgtatgagccctgagtcctacctgggctccccccagcatagcccctccacctccaggggatcaccaagcagtctgccctctccagttgttacccgtgggtcaccaagacccaaaccttatgacccccctggagttactttaacagctaaagtgaaaattgaaaagttggataagaagctaaaaaaaatggagcaaaacaagacagcagccactagataccgacagaagaagcgggctgaacaggaagccctgacaggcgagtgtagagagctagaaaagaagaatgaagctctaaaagagaaggcagattctcttgccaaagagatccaatatctgaaagatctgatagaagaggtccggaaggcaagggggaagaagagagctccctag